European Patent Specification EP 3 448 423 B1, published July 19, 2023. Title: A therapeutic inhibitor for EBV-associated tumor with tailor responsive optical imaging. Applicant: Hong Kong Baptist University. The sequence listing filed with the application follows.

SEQUENCE LISTING (4 sequences)

SEQ ID NO: 1 - protein, 5 aa, Artificial sequence
  The sequence is synthesized
YFMVF

SEQ ID NO: 2 - protein, 13 aa, Artificial sequence
  The sequence is synthesized
  PEPTIDE (2)..(2): X is 6-aminohexanoic acid
  PEPTIDE (3)..(3): R is L-arginine
  PEPTIDE (4)..(4): X is D-arginine
  PEPTIDE (5)..(5): R is L-arginine
CXRXRKGGYFMVF

SEQ ID NO: 3 - protein, 13 aa, Artificial sequence
  The sequence is synthesized
  PEPTIDE (2)..(2): X is 6-aminohexanoic acid
  PEPTIDE (10)..(10): R is L-arginine
  PEPTIDE (11)..(11): X is D-arginine
  PEPTIDE (12)..(12): R is L-arginine
CXYFMVFGGRXRK

SEQ ID NO: 4 - protein, 147 aa, Human Gamma Herpes Virus 4
KGGWFGKHRGQGGSNPKFENIAEGLRALLARSHVERTTDEGTWVAGVFVYGGSKTSLYNLRRGTALAIPQCRLTPLSRLPFGMAPGPGPQPGPLRESIVCYFMVFLQTHIFAEVLKDAIKDLVMTKPAPTCNIRVTVCSFDDGVDLP